European Patent Application EP 4 137 508 A1, published February 22, 2023. Title: Variants of Ankyrin Repeat Domains. Applicant: Athebio AG. The sequence listing filed with the application follows.

SEQUENCE LISTING (84 sequences)

SEQ ID NO: 1 - protein, 30 aa, Artificial Sequence
  Synthetic construct
DLGKKLLEAARAGQDDEVRILMANGADVNA

SEQ ID NO: 2 - protein, 30 aa, Artificial Sequence
  Synthetic construct
DLGKKLLEAARAGQDDEVRELLKAGADVNA

SEQ ID NO: 3 - protein, 30 aa, Artificial Sequence
  Synthetic construct
DLGKKLLEAARAGQDDEVRILLKAGADVNA

SEQ ID NO: 4 - protein, 30 aa, Artificial Sequence
  Synthetic construct
DLDKKLLEAARAGQDDEVRILMANGADVNA

SEQ ID NO: 5 - protein, 30 aa, Artificial Sequence
  Synthetic construct
DLGKKLLEAARAGQDDEVRILIANGAPFTT

SEQ ID NO: 6 - protein, 30 aa, Artificial Sequence
  Synthetic construct
DLGKKLLEAARAGQDDEVRELTKAGADVNA

SEQ ID NO: 7 - protein, 30 aa, Artificial Sequence
  Synthetic construct
DLGKKLLEAARAGQDDEVHILIANGADVNA

SEQ ID NO: 8 - protein, 30 aa, Artificial Sequence
  Synthetic construct
DLGKKLLQAARAGQLDEVRELLKAGADVNA

SEQ ID NO: 9 - protein, 30 aa, Artificial Sequence
  Synthetic construct
DLGKKLLKAARAGQKDEVKILMENGADVNA

SEQ ID NO: 10 - protein, 30 aa, Artificial Sequence
  Synthetic construct
DLGKKLLEAARAGQDDEVRILMALGADVNA

SEQ ID NO: 11 - protein, 30 aa, Artificial Sequence
  Synthetic construct
DLGKKLLEAARAGQIDEVRELLKLGADVNA

SEQ ID NO: 12 - protein, 30 aa, Artificial Sequence
  Synthetic construct
DLDKKLLEAARAGQLDEVRELTKLGADVNA

SEQ ID NO: 13 - protein, 30 aa, Artificial Sequence
  Synthetic construct
DLGKKLLEAARAGQVDEVRELIKLGADVNA

SEQ ID NO: 14 - protein, 30 aa, Artificial Sequence
  Synthetic construct
DLDKKLLEAAAAGQIDAVRELLKLGADVNA

SEQ ID NO: 15 - protein, 30 aa, Artificial Sequence
  Synthetic construct
DLAKKLLEAAAAGQLDAVRELVKLGADVNA

SEQ ID NO: 16 - protein, 30 aa, Artificial Sequence
  Synthetic construct
DLGKKLLEAAAAGQVDAVRELIKLGADVNA

SEQ ID NO: 17 - protein, 30 aa, Artificial Sequence
  Synthetic construct
DLAKKLLEAAAAGQIDAVRELAKLGADVNA

SEQ ID NO: 18 - protein, 30 aa, Artificial Sequence
  Synthetic construct
DLAKKLLAAAAAGQLEAVEQLLKLGADVNA

SEQ ID NO: 19 - protein, 30 aa, Artificial Sequence
  Synthetic construct
DLGKKLLAAAAAGQVEAVEQLIKLGADVNA

SEQ ID NO: 20 - protein, 30 aa, Artificial Sequence
  Synthetic construct
DLGKKLLEAAAAGQLDEVRILIALGADVNA

SEQ ID NO: 21 - protein, 30 aa, Artificial Sequence
  Synthetic construct
DLGKKLLEAAAAGQLDEVKELIALGADVNA

SEQ ID NO: 22 - protein, 30 aa, Artificial Sequence
  Synthetic construct
DLGKKLLEAARAGQLDEVRELLKLGADVNA

SEQ ID NO: 23 - protein, 30 aa, Artificial Sequence
  Synthetic construct
DLGKKLLEAAEAGQVDEVKELLKLGADVNA

SEQ ID NO: 24 - protein, 30 aa, Artificial Sequence
  Synthetic construct
DLGKKLLEAARAGQLDEVRILLKLGADVNA

SEQ ID NO: 25 - protein, 30 aa, Artificial Sequence
  Synthetic construct
DLGKKLLEAAEAGQVDEVKILLKLGADVNA

SEQ ID NO: 26 - protein, 30 aa, Artificial Sequence
  Synthetic construct
DLGKKLLEAAAAGQVDEVRELIKLGADVNA

SEQ ID NO: 27 - protein, 30 aa, Artificial Sequence
  Synthetic construct
DLGKKLLEAAAAGQVDEVKELIKLGADVNA

SEQ ID NO: 28 - protein, 30 aa, Artificial Sequence
  Synthetic construct
DLGKKLLEAARAGQLDEVRILIKLGADVNA

SEQ ID NO: 29 - protein, 30 aa, Artificial Sequence
  Synthetic construct
DLGKKLLEAARAGQLDEVKILIKLGADVNA

SEQ ID NO: 30 - protein, 30 aa, Artificial Sequence
  Synthetic construct
DLGKKLLEAAEAGQLDEVRELLALGADVNA

SEQ ID NO: 31 - protein, 30 aa, Artificial Sequence
  Synthetic construct
DLGKKLLEAAEAGQLDEVKELLALGADVNA

SEQ ID NO: 32 - protein, 30 aa, Artificial Sequence
  Synthetic construct
DLGKKLLEAAAAGQVDEVKELIALGADVNA

SEQ ID NO: 33 - protein, 30 aa, Artificial Sequence
  Synthetic construct
DLGKKLLEAARAGQIDEVKILLALGADVNA

SEQ ID NO: 34 - protein, 30 aa, Artificial Sequence
  Synthetic construct
DLGKKLLEAAAAGQIDEVRELIALGADVNA

SEQ ID NO: 35 - protein, 30 aa, Artificial Sequence
  Synthetic construct
DLGKKLLEAAAAGQIDEVKELIALGADVNA

SEQ ID NO: 36 - protein, 30 aa, Artificial Sequence
  Synthetic construct
DLGKKLLEAAEAGQIDEVRILIALGADVNA

SEQ ID NO: 37 - protein, 30 aa, Artificial Sequence
  Synthetic construct
DLGKKLLEAAEAGQIDEVKILIALGADVNA

SEQ ID NO: 38 - protein, 30 aa, Artificial Sequence
  Synthetic construct
  VARIANT 1: Xaa is selected from the group consisting of G, D, A, E, N, Q, S, T, K, R, H and C
  VARIANT 2: Xaa is selected from the group consisting of L, Q, E, M, K, R and C
  VARIANT 3: Xaa is selected from the group consisting of G, A, D, S and C
  VARIANT 4: Xaa is selected from the group consisting of Q, N, S, T, A, D, E, K, R, H and C
  VARIANT 5: Xaa is selected from the group consisting of Q, N, S, T, A, D, E, K, R, H and C
  VARIANT 6: Xaa is selected from the group consisting of L, A, N, S, D and C
  VARIANT 7: Xaa is selected from the group consisting of L, I, V, A, N, T, S, D and C
  VARIANT 8: Xaa is selected from the group consisting of Q, N, S, T, A, D, E, K, R, H and C
  VARIANT 10: Xaa is selected from the group consisting of A, V, S and C
  VARIANT 11: Xaa is selected from the group consisting of R, A, L, S, Q, K, H, D, E, C, T, N, F, W and Y
  VARIANT 12: Xaa is selected from the group consisting of Q, N, S, T, A, D, E, K, R, H and C
  VARIANT 13: Xaa is selected from the group consisting of G and C
  VARIANT 14: Xaa is selected from the group consisting of Q, N, S, T, A, D, E, K, R, H and C
  VARIANT 15: Xaa is selected from the group consisting of D, L, M, I, T, A, V, S, N, Q, K, R, E and C
  VARIANT 16: Xaa is selected from the group consisting of Q, N, S, T, A, D, E, K, R, H and C
  VARIANT 17: Xaa is selected from the group consisting of Q, N, S, T, A, D, E, K, R, H and C
  VARIANT 18: Xaa is selected from the group consisting of L, I, V, T, A, S and C
  VARIANT 19: Xaa is selected from the group consisting of Q, N, S, T, A, D, E, K, R, H and C
  VARIANT 20: Xaa is selected from the group consisting of E, Q, N, K, R, A, D, T, S, H, I, V and C
  VARIANT 21: Xaa is selected from the group consisting of L, N, S, A and C
  VARIANT 22: Xaa is selected from the group consisting of L, I, A, V, M, T, S, N and C
  VARIANT 23: Xaa is selected from the group consisting of K, R, S, Q, N, A, E, D, H and C
  VARIANT 24: Xaa is selected from the group consisting of A, K, R, H, L, I, V, C and G
  VARIANT 27: Xaa is selected from the group consisting of D, N and C
  VARIANT 28: Xaa is selected from the group consisting of V, T, S, P, A and C
  VARIANT 29: Xaa is selected from the group consisting of N, D and C
  VARIANT 30: Xaa is selected from the group consisting of A and C
XXXXXXXXAXXXXXXXXXXXXXXXGAXXXX

SEQ ID NO: 39 - protein, 33 aa, Artificial Sequence
  Synthetic construct
  VARIANT 1: Xaa can be any amino acid residue
  VARIANT 3: Xaa can be any amino acid residue
  VARIANT 4: Xaa can be any amino acid residue
  VARIANT 6: Xaa can be any amino acid residue
  VARIANT 13: Xaa can be any amino acid residue
  VARIANT 14: Xaa can be any amino acid residue
  VARIANT 15: Xaa can be any amino acid residue
  VARIANT 17: Xaa can be any amino acid residue
  VARIANT 18: Xaa can be any amino acid residue
  VARIANT 19: Xaa can be any amino acid residue
  VARIANT 22: Xaa can be any amino acid residue
  VARIANT 26: Xaa can be any amino acid residue
  VARIANT 27: Xaa can be any amino acid residue
XDXXGXTPLHLAXXXGXXXVVXLLLXXGADVNA

SEQ ID NO: 40 - protein, 33 aa, Artificial Sequence
  Synthetic construct
  VARIANT 1: Xaa can be any amino acid residue
  VARIANT 3: Xaa can be any amino acid residue
  VARIANT 4: Xaa can be any amino acid residue
  VARIANT 6: Xaa can be any amino acid residue
  VARIANT 14: Xaa can be any amino acid residue
  VARIANT 15: Xaa can be any amino acid residue
  VARIANT 27: Xaa can be any amino acid residue
XDXXGXTPLHLAAXXGHLEIVEVLLKXGADVNA

SEQ ID NO: 41 - protein, 33 aa, Artificial Sequence
  Synthetic construct
  VARIANT 2: Xaa can be any amino acid residue
  VARIANT 3: Xaa can be any amino acid residue
  VARIANT 4: Xaa can be any amino acid residue
  VARIANT 6: Xaa can be any amino acid residue
  VARIANT 11: Xaa can be any amino acid residue
  VARIANT 14: Xaa can be any amino acid residue
  VARIANT 15: Xaa can be any amino acid residue
  VARIANT 27: Xaa can be any amino acid residue
SXXXGXTPLHXAAXXGHLEIVDVLLAXGADVNA

SEQ ID NO: 42 - protein, 33 aa, Artificial Sequence
  Synthetic construct
  VARIANT 1: Xaa can be any amino acid residue
  VARIANT 3: Xaa can be any amino acid residue
  VARIANT 4: Xaa can be any amino acid residue
  VARIANT 6: Xaa can be any amino acid residue
  VARIANT 14: Xaa can be any amino acid residue
  VARIANT 15: Xaa can be any amino acid residue
XDXXGXTPLHLAAXXGHLEIVEVLLKNGADVNA

SEQ ID NO: 43 - protein, 33 aa, Artificial Sequence
  Synthetic construct
  VARIANT 3: Xaa can be any amino acid residue
  VARIANT 4: Xaa can be any amino acid residue
  VARIANT 6: Xaa can be any amino acid residue
  VARIANT 14: Xaa can be any amino acid residue
  VARIANT 15: Xaa can be any amino acid residue
KDXXGXTPLHLAAXXGHLEIVEVLLKAGADVNA

SEQ ID NO: 44 - protein, 33 aa, Artificial Sequence
  Synthetic construct
  VARIANT 1: Xaa can be any amino acid residue
  VARIANT 3: Xaa can be any amino acid residue
  VARIANT 4: Xaa can be any amino acid residue
  VARIANT 6: Xaa can be any amino acid residue
  VARIANT 11: Xaa can be any amino acid residue
  VARIANT 14: Xaa can be any amino acid residue
  VARIANT 15: Xaa can be any amino acid residue
  VARIANT 27: Xaa can be any amino acid residue
XDXXGXTPLHXAAXXGHLEVVKLLLEXGADVNA

SEQ ID NO: 45 - protein, 33 aa, Artificial Sequence
  Synthetic Construct
  VARIANT 1: Xaa can be any amino acid residue
  VARIANT 3: Xaa can be any amino acid residue
  VARIANT 4: Xaa can be any amino acid residue
  VARIANT 6: Xaa can be any amino acid residue
  VARIANT 14: Xaa can be any amino acid residue
  VARIANT 15: Xaa can be any amino acid residue
XDXXGXTPLHLAAXXGHLEIVKLLLEAGADVNA

SEQ ID NO: 46 - protein, 33 aa, Artificial Sequence
  Synthetic Construct
  VARIANT 1: Xaa can be any amino acid residue
  VARIANT 3: Xaa can be any amino acid residue
  VARIANT 4: Xaa can be any amino acid residue
  VARIANT 6: Xaa can be any amino acid residue
  VARIANT 14: Xaa can be any amino acid residue
  VARIANT 15: Xaa can be any amino acid residue
XDXXGXTPLHLAAXXGHIEIVELLLKAGADVNA

SEQ ID NO: 47 - protein, 28 aa, Artificial Sequence
  Synthetic construct
QDKFGKTAFDISIDNGNEDLAEILQKLN

SEQ ID NO: 48 - protein, 28 aa, Artificial Sequence
  Synthetic construct
QDKFGKTAFDISIDNGNEDLAEILQKAA

SEQ ID NO: 49 - protein, 28 aa, Artificial Sequence
  Synthetic construct
QDKFGKTPFDLAIDNGNEDIAEVLQKAA

SEQ ID NO: 50 - protein, 28 aa, Artificial Sequence
  Synthetic construct
QDKFGKTPFDLAIREGHEDIAEVLQKAA

SEQ ID NO: 51 - protein, 28 aa, Artificial Sequence
  Synthetic construct
QDKSGKTPADLAADAGHEDIAEVLQKAA

SEQ ID NO: 52 - protein, 28 aa, Artificial Sequence
  Synthetic construct
QDSAGKTPADLAADAGHEEIAEVLQKAA

SEQ ID NO: 53 - protein, 28 aa, Artificial Sequence
  Synthetic construct
QDKAGLTPADLAADAGHEEIAEVLQKAA

SEQ ID NO: 54 - protein, 28 aa, Artificial Sequence
  Synthetic construct
QDSLGKTPADLAALAGHEEIAEVLQKAA

SEQ ID NO: 55 - protein, 28 aa, Artificial Sequence
  Synthetic construct
QDKAGQTPADLAADAGHEEIAEVLQKAA

SEQ ID NO: 56 - protein, 28 aa, Artificial Sequence
  Synthetic construct
  VARIANT 3: Xaa can be any amino acid residue
  VARIANT 4: Xaa can be any amino acid residue
  VARIANT 6: Xaa can be any amino acid residue
  VARIANT 14: Xaa can be any amino acid residue
QDXXGXTPADLAAXAGHEEIAEVLQKAA

SEQ ID NO: 57 - protein, 28 aa, Artificial Sequence
  Synthetic construct
QDKSGKTPADLAARAGHQDIAEVLQKAA

SEQ ID NO: 58 - protein, 28 aa, Artificial Sequence
  Synthetic construct
QDKFGKTAEDLAKDNGNQDIADLLEKAL

SEQ ID NO: 59 - protein, 27 aa, Artificial Sequence
  Synthetic construct
QDKFGKTAFDISIDNGNEELAKVLQDH

SEQ ID NO: 60 - protein, 103 aa, Artificial Sequence
  Synthetic construct
MRGSHHHHHHGSDLGKKLLEAAAAGQLDEVKELIAAGADVNAKDKDGYTPLHLAAREGHLEIVEVLLKAGADVNAQDKFGKTAFDISIDNGNEDLAEILQKLN

SEQ ID NO: 61 - protein, 103 aa, Artificial Sequence
  Synthetic construct
MRGSHHHHHHGSDLGKKLLEAAAAGQLDEVKELIALGADVNAKDKDGYTPLHLAAREGHLEIVEVLLKAGADVNAQDKFGKTAFDISIDNGNEDLAEILQKLN

SEQ ID NO: 62 - protein, 103 aa, Artificial Sequence
  Synthetic construct
MRGSHHHHHHGSDLGKKLLEAAAAGQLDEVKELIAGGADVNAKDKDGYTPLHLAAREGHLEIVEVLLKAGADVNAQDKFGKTAFDISIDNGNEDLAEILQKLN

SEQ ID NO: 63 - protein, 103 aa, Artificial Sequence
  Synthetic construct
MRGSHHHHHHGSDLGKKLLEAAAAGQLDEVKELIAVGADVNAKDKDGYTPLHLAAREGHLEIVEVLLKAGADVNAQDKFGKTAFDISIDNGNEDLAEILQKLN

SEQ ID NO: 64 - protein, 103 aa, Artificial Sequence
  Synthetic construct
MRGSHHHHHHGSDLGKKLLEAAAAGQLDEVKELIAEGADVNAKDKDGYTPLHLAAREGHLEIVEVLLKAGADVNAQDKFGKTAFDISIDNGNEDLAEILQKLN

SEQ ID NO: 65 - protein, 103 aa, Artificial Sequence
  Synthetic construct
MRGSHHHHHHGSDLGKKLLEAAAAGQLDEVKELIANGADVNAKDKDGYTPLHLAAREGHLEIVEVLLKAGADVNAQDKFGKTAFDISIDNGNEDLAEILQKLN

SEQ ID NO: 66 - protein, 103 aa, Artificial Sequence
  Synthetic construct
MRGSHHHHHHGSDLGKKLLEAAAAGQLDEVKELIAQGADVNAKDKDGYTPLHLAAREGHLEIVEVLLKAGADVNAQDKFGKTAFDISIDNGNEDLAEILQKLN

SEQ ID NO: 67 - protein, 103 aa, Artificial Sequence
  Synthetic construct
MRGSHHHHHHGSDLGKKLLEAAAAGQLDEVKELIASGADVNAKDKDGYTPLHLAAREGHLEIVEVLLKAGADVNAQDKFGKTAFDISIDNGNEDLAEILQKLN

SEQ ID NO: 68 - protein, 136 aa, Artificial Sequence
  Synthetic construct
MRGSHHHHHHGSDLGKKLLEAARAGQDDEVRELLKAGADVNAKDYFSHTPLHLAARNGHLKIVEVLLKAGADVNAKDFAGKTPLHLAANEGHLEIVEVLLKAGADVNAQDIFGKTPADIAADAGHEDIAEVLQKAA

SEQ ID NO: 69 - protein, 136 aa, Artificial Sequence
  Synthetic construct
MRGSHHHHHHGSDLGKKLLEAARAGQDDEVRELLKLGADVNAKDYFSHTPLHLAARNGHLKIVEVLLKAGADVNAKDFAGKTPLHLAANEGHLEIVEVLLKAGADVNAQDIFGKTPADIAADAGHEDIAEVLQKAA

SEQ ID NO: 70 - protein, 136 aa, Artificial Sequence
  Synthetic construct
MRGSHHHHHHGSDLDKKLLEAARAGQDDEVRILMANGADVNARDSTGWTPLHLAAPWGHPEIVEVLLKNGADVNAADFQGWTPLHLAAAVGHLEIVEVLLKYGADVNAQDKFGKTAFDISIDNGNEDLAEILQKAA

SEQ ID NO: 71 - protein, 136 aa, Artificial Sequence
  Synthetic construct
MRGSHHHHHHGSDLDKKLLEAARAGQDDEVRILMALGADVNARDSTGWTPLHLAAPWGHPEIVEVLLKNGADVNAADFQGWTPLHLAAAVGHLEIVEVLLKYGADVNAQDKFGKTAFDISIDNGNEDLAEILQKAA

SEQ ID NO: 72 - protein, 136 aa, Artificial Sequence
  Synthetic construct
MRGSHHHHHHGSDLGKKLLEAARAGQDDEVRILMANGADVNAKDEYGLTPLYLATAHGHLEIVEVLLKNGADVNAVDAIGFTPLHLAAFIGHLEIAEVLLKHGADVNAQDKFGKTAFDISIGNGNEDLAEILQKLN

SEQ ID NO: 73 - protein, 136 aa, Artificial Sequence
  Synthetic construct
MRGSHHHHHHGSDLGKKLLEAARAGQDDEVRILMALGADVNAKDEYGLTPLYLATAHGHLEIVEVLLKNGADVNAVDAIGFTPLHLAAFIGHLEIAEVLLKHGADVNAQDKFGKTAFDISIGNGNEDLAEILQKLN

SEQ ID NO: 74 - protein, 169 aa, Artificial Sequence
  Synthetic construct
MRGSHHHHHHGSDLGKKLLQAARAGQLDEVRELLKAGADVNAKDREGITPLHLAAQHGHLEIVEVLLKAGADVNAKDVWGRTPLHLAAQWGHLEIVEVLLKAGADVNAKDLAGATPLHVAALYGHLEIVEVLLKAGADVNAQDKSGKTPADLAARAGHQDIAEVLQKAA

SEQ ID NO: 75 - protein, 169 aa, Artificial Sequence
  Synthetic construct
MRGSHHHHHHGSDLGKKLLQAARAGQLDEVRELLKLGADVNAKDREGITPLHLAAQHGHLEIVEVLLKAGADVNAKDVWGRTPLHLAAQWGHLEIVEVLLKAGADVNAKDLAGATPLHVAALYGHLEIVEVLLKAGADVNAQDKSGKTPADLAARAGHQDIAEVLQKAA

SEQ ID NO: 76 - protein, 136 aa, Artificial Sequence
  Synthetic construct
MRGSHHHHHHGSDLGKKLLEAAAAGQDDEVKELIALGADVNAKDYFSHTPLHLAARNGHLKIVEVLLKAGADVNAKDFAGKTPLHLAANEGHLEIVEVLLKAGADVNAQDIFGKTPADIAADAGHEDIAEVLQKAA

SEQ ID NO: 77 - protein, 136 aa, Artificial Sequence
  Synthetic construct
MRGSHHHHHHGSDLGKKLLEAAAAGQLDEVKELIALGADVNAKDYFSHTPLHLAARNGHLKIVEVLLKAGADVNAKDFAGKTPLHLAANEGHLEIVEVLLKAGADVNAQDIFGKTPADIAADAGHEDIAEVLQKAA

SEQ ID NO: 78 - protein, 136 aa, Artificial Sequence
  Synthetic construct
MRGSHHHHHHGSDLGKKLLEAAAAGQVDEVKELIALGADVNAKDYFSHTPLHLAARNGHLKIVEVLLKAGADVNAKDFAGKTPLHLAANEGHLEIVEVLLKAGADVNAQDIFGKTPADIAADAGHEDIAEVLQKAA

SEQ ID NO: 79 - protein, 136 aa, Artificial Sequence
  Synthetic construct
MRGSHHHHHHGSDLGKKLLEAAAAGQIDEVKELIALGADVNAKDYFSHTPLHLAARNGHLKIVEVLLKAGADVNAKDFAGKTPLHLAANEGHLEIVEVLLKAGADVNAQDIFGKTPADIAADAGHEDIAEVLQKAA

SEQ ID NO: 80 - protein, 103 aa, Artificial Sequence
  Synthetic construct
MRGSHHHHHHGSDLGKKLLEAARAGQLDEVKELIAAGADVNAKDKDGYTPLHLAAREGHLEIVEVLLKAGADVNAQDKFGKTAFDISIDNGNEDLAEILQKLN

SEQ ID NO: 81 - protein, 103 aa, Artificial Sequence; identical to SEQ ID NO: 60
  Synthetic construct

SEQ ID NO: 82 - protein, 103 aa, Artificial Sequence
  Synthetic construct
MRGSHHHHHHGSDLGKKLLEAAKAGQLDEVKELIAAGADVNAKDKDGYTPLHLAAREGHLEIVEVLLKAGADVNAQDKFGKTAFDISIDNGNEDLAEILQKLN

SEQ ID NO: 83 - protein, 103 aa, Artificial Sequence
  Synthetic construct
MRGSHHHHHHGSDLGKKLLEAAEAGQLDEVKELIAAGADVNAKDKDGYTPLHLAAREGHLEIVEVLLKAGADVNAQDKFGKTAFDISIDNGNEDLAEILQKLN

SEQ ID NO: 84 - protein, 103 aa, Artificial Sequence
  Synthetic construct
MRGSHHHHHHGSDLGKKLLEAAQAGQLDEVKELIAAGADVNAKDKDGYTPLHLAAREGHLEIVEVLLKAGADVNAQDKFGKTAFDISIDNGNEDLAEILQKLN